European Patent Specification EP 3 563 863 B1, published July 12, 2023. Title: Lyophilized Preparation. Applicant: JCR Pharmaceuticals Co., Ltd. The sequence listing filed with the application follows.

SEQUENCE LISTING (61 sequences)

SEQ ID NO: 1 - protein, 525 aa, Homo sapiens
SETQANSTTDALNVLLIIVDDLRPSLGCYGDKLVRSPNIDQLASHSLLFQNAFAQQAVCAPSRVSFLTGRRPDTTRLYDFNSYWRVHAGNFSTIPQYFKENGYVTMSVGKVFHPGISSNHTDDSPYSWSFPPYHPSSEKYENTKTCRGPDGELHANLLCPVDVLDVPEGTLPDKQSTEQAIQLLEKMKTSASPFFLAVGYHKPHIPFRYPKEFQKLYPLENITLAPDPEVPDGLPPVAYNPWMDIRQREDVQALNISVPYGPIPVDFQRKIRQSYFASVSYLDTQVGRLLSALDDLQLANSTIIAFTSDHGWALGEHGEWAKYSNFDVATHVPLIFYVPGRTASLPEAGEKLFPYLDPFDSASQLMEPGRQSMDLVELVSLFPTLAGLAGLQVPPRCPVPSFHVELCREGKNLLKHFRFRDLEEDPYLPGNPRELIAYSQYPRPSDIPQWNSDKPSLKDIKIMGYSIRTIDYRYTVWVGFNPDEFLANFSDIHAGELYFVDSDPLQDHNMYNDSQGGDLFQLLMP

SEQ ID NO: 2 - protein, 214 aa, Artificial Sequence
  Amino acid sequence of the light-chain of humanized anti-hTfR antibody No. 1
DIQVTQSPSFLSASVGDRVTITCKASQDVNSAVAWFQQKPGKAPKLLIYWTSTRHTGVPDRFSGSGSGTVYTLTISSLQPEDFATYYCQQHYSTPRTFGGGTKVEIKRTVAAPSVFIFPPSDEQLKSGTASVVCLLNNFYPREAKVQWKVDNALQSGNSQESVTEQDSKDSTYSLSSTLTLSKADYEKHKVYACEVTHQGLSSPVTKSFNRGEC

SEQ ID NO: 3 - DNA, 725 bp, Artificial Sequence
  Nucleotide seuquence encoding amino acid sequence of the light-chain of humanized anti-hTfR antibody No. 1, synthetic sequence
acgcgtgccgccaccatgggctggagctggattctgctgttcctcctgagcgtgacagcaggagtgcacagcgacatccaggtcacacagtcaccaagttttctgagcgcaagcgtgggcgacagggtcactatcacatgcaaggcaagccaggacgtgaactccgcagtggcctggttccagcagaagccagggaaagcacccaagctgctgatctattggacctctacaaggcacaccggtgtcccagatcggttctcaggttccggcagcggaacagtgtatactctgaccatttccagcctgcagcctgaagacttcgctacttactattgccagcagcattactccaccccaagaacatttggcggagggactaaagtggagatcaagaggaccgtggccgctccctccgtcttcatttttccccctagcgacgaacagctgaagagtggcacagcctcagtggtctgtctgctgaacaatttctaccctagggaggctaaagtgcagtggaaggtcgataacgcactgcagtctggaaatagtcaggagtcagtgacagaacaggactccaaagatagcacttattctctgtctagtacactgactctgagcaaggccgattacgaaaagcacaaagtgtatgcttgcgaagtcacccatcaggggctgtcatcaccagtcaccaagtcattcaatagaggcgagtgctaagcggccgc

SEQ ID NO: 4 - protein, 214 aa, Artificial Sequence
  Amino acid sequence of the light-chain of humanized anti-hTfR antibody No. 2
EIVLTQSPDFQSVTPKEKVTITCRASQSISNNLQWYQQKPDQSPKLLIKYASQSISGIPSRFSGSGSGTDFTLTINSLEAEDAATYLCQQSNSWPRTFGQGTKVEIKRTVAAPSVFIFPPSDEQLKSGTASVVCLLNNFYPREAKVQWKVDNALQSGNSQESVTEQDSKDSTYSLSSTLTLSKADYEKHKVYACEVTHQGLSSPVTKSFNRGEC

SEQ ID NO: 5 - DNA, 725 bp, Artificial Sequence
  Nucleotide seuquence encoding amino acid sequence of the light-chain of humanized anti-hTfR antibody No. 2, synthetic sequence
acgcgtgccgccaccatgggctggagctggattctgctgttcctcctgagcgtgacagcaggagtgcacagcgaaattgtgctgacccagtctcccgatttccagtccgtgacccccaaggagaaagtcaccatcacatgcagagcatcacagtccattagcaacaatctgcagtggtaccagcagaagccagaccagagccccaagctgctgatcaaatatgcctctcagagtatttcaggcataccttctaggttctccggtagcggctctggaaccgactttactctgaccatcaacagtctggaggctgaagatgccgctacatacttgtgccagcagagtaattcatggcctaggacctttggccaggggacaaaggtggagatcaaaaggactgtggcagccccaagtgtcttcatttttcccccttcagacgaacagctgaagagcggcacagcatctgtggtctgtctgctgaacaatttctacccacgggaggctaaggtgcagtggaaagtcgataacgcactgcagtccggaaatagccaggagtctgtgactgaacaggacagtaaggattcaacctattccctgtccagcacactgactctgagcaaagccgattacgagaagcacaaagtgtatgcttgcgaagtcacacatcaggggctgtctagtcccgtgactaagtcttttaataggggtgaatgttaagcggccgc

SEQ ID NO: 6 - protein, 219 aa, Artificial Sequence
  amino acid sequence of the light-chain of humanized anti-hTfR antibody No. 3
DIVMTQTPLSLSVTPGQPASISCRSSQSLVHSNGNTYLHWYLQKPGQSPQLLIYKVSNRFSGVPDRFSGSGSGTDFTLKISRVEAEDVGVYYCSQSTHVPWTFGQGTKVEIKRTVAAPSVFIFPPSDEQLKSGTASVVCLLNNFYPREAKVQWKVDNALQSGNSQESVTEQDSKDSTYSLSSTLTLSKADYEKHKVYACEVTHQGLSSPVTKSFNRGEC

SEQ ID NO: 7 - DNA, 740 bp, Artificial Sequence
  Nucleotide seuquence encoding amino acid sequence of the light-chain of humanized anti-hTfR antibody No. 3, synthetic sequence
acgcgtgccgccaccatgggctggagctggattctgctgttcctcctgagcgtgacagcaggagtgcacagcgacatcgtgatgacccagactcccctgagcctgagcgtgacacctggccagcctgccagcatcagctgcagaagctctcagagcctggtgcacagcaacggcaacacctacctgcactggtatctgcagaagcccggccagagccctcagctgctgatctacaaggtgtccaacagattcagcggcgtgcccgacagattctccggcagcggctctggcaccgacttcaccctgaagatttccagagtggaagccgaggacgtgggcgtgtactactgcagccagagcacccacgtgccctggacattcggccagggcaccaaggtggaaatcaagagaaccgtggccgctcccagcgtgttcatcttcccacctagcgacgagcagctgaagtccggcacagcctctgtcgtgtgcctgctgaacaacttctacccccgcgaggccaaggtgcagtggaaggtggacaacgccctgcagagcggcaacagccaggaaagcgtgaccgagcaggactccaaggacagcacctacagcctgagcagcaccctgaccctgagcaaggccgactacgagaagcacaaggtgtacgcctgcgaagtgacccaccagggcctgtctagccccgtgaccaagagcttcaacagaggcgagtgctaagcggccgc

SEQ ID NO: 8 - protein, 446 aa, Artificial Sequence
  Amino acid sequence of the heavy-chain of humanized anti-hTfR antibody No. 1
EVQLVESGGGLVQPGGSLRLSCAASGLTFSNYGMSWVRQAPGKGLELVANINTNGGSTYYPDSVKGRFTISRDNAKNSLYLQMNSLRAEDTAVYYCTNNRYDEDYWGQGTLVTVSSASTKGPSVFPLAPSSKSTSGGTAALGCLVKDYFPEPVTVSWNSGALTSGVHTFPAVLQSSGLYSLSSVVTVPSSSLGTQTYICNVNHKPSNTKVDKKVEPKSCDKTHTCPPCPAPELLGGPSVFLFPPKPKDTLMISRTPEVTCVVVDVSHEDPEVKFNWYVDGVEVHNAKTKPREEQYNSTYRVVSVLTVLHQDWLNGKEYKCKVSNKALPAPIEKTISKAKGQPREPQVYTLPPSRDELTKNQVSLTCLVKGFYPSDIAVEWESNGQPENNYKTTPPVLDSDGSFFLYSKLTVDKSRWQQGNVFSCSVMHEALHNHYTQKSLSLSPGK

SEQ ID NO: 9 - protein, 453 aa, Artificial Sequence
  Amino acid sequence of the heavy-chain of humanized anti-hTfR antibody No. 2
QVQLVQSGAEVKKPGASVKVSCKASGYTFTDYVMHWVRQAPGQGLEWIGVISTYYGHGSYNQRFKGRATMTVDKSISTAYMELVRLRSDDTAVYYCVRGGYGSSSLAGNFDVWGQGTTVTVSSASTKGPSVFPLAPSSKSTSGGTAALGCLVKDYFPEPVTVSWNSGALTSGVHTFPAVLQSSGLYSLSSVVTVPSSSLGTQTYICNVNHKPSNTKVDKKVEPKSCDKTHTCPPCPAPELLGGPSVFLFPPKPKDTLMISRTPEVTCVVVDVSHEDPEVKFNWYVDGVEVHNAKTKPREEQYNSTYRVVSVLTVLHQDWLNGKEYKCKVSNKALPAPIEKTISKAKGQPREPQVYTLPPSRDELTKNQVSLTCLVKGFYPSDIAVEWESNGQPENNYKTTPPVLDSDGSFFLYSKLTVDKSRWQQGNVFSCSVMHEALHNHYTQKSLSLSPGK

SEQ ID NO: 10 - protein, 448 aa, Artificial Sequence
  Amino acid sequence of the heavy-chain of humanized anti-hTfR antibody No. 3
EVQLVQSGAEVKKPGESLKISCKGSGYSFTNYWLGWVRQMPGKGLEWMGDIYPGGDYPTYSEKFKVQVTISADKSISTAYLQWSSLKASDTAMYYCARSGNYDEVAYWGQGTLVTVSSASTKGPSVFPLAPSSKSTSGGTAALGCLVKDYFPEPVTVSWNSGALTSGVHTFPAVLQSSGLYSLSSVVTVPSSSLGTQTYICNVNHKPSNTKVDKKVEPKSCDKTHTCPPCPAPELLGGPSVFLFPPKPKDTLMISRTPEVTCVVVDVSHEDPEVKFNWYVDGVEVHNAKTKPREEQYNSTYRVVSVLTVLHQDWLNGKEYKCKVSNKALPAPIEKTISKAKGQPREPQVYTLPPSRDELTKNQVSLTCLVKGFYPSDIAVEWESNGQPENNYKTTPPVLDSDGSFFLYSKLTVDKSRWQQGNVFSCSVMHEALHNHYTQKSLSLSPGK

SEQ ID NO: 11 - DNA, 20 bp, Artificial Sequence
  Primer Hyg-Sfi5', synthetic sequence
gaggccgcctcggcctctga

SEQ ID NO: 12 - DNA, 29 bp, Artificial Sequence
  Primer Hyg-BstX3', synthetic sequence
aaccatcgtgatgggtgctattcctttgc

SEQ ID NO: 13 - protein, 973 aa, Artificial Sequence
  Amino acid sequence of fused protein of the heavy-chain of humanized anti-hTfR antibody No.1 and hI2S
EVQLVESGGGLVQPGGSLRLSCAASGLTFSNYGMSWVRQAPGKGLELVANINTNGGSTYYPDSVKGRFTISRDNAKNSLYLQMNSLRAEDTAVYYCTNNRYDEDYWGQGTLVTVSSASTKGPSVFPLAPSSKSTSGGTAALGCLVKDYFPEPVTVSWNSGALTSGVHTFPAVLQSSGLYSLSSVVTVPSSSLGTQTYICNVNHKPSNTKVDKKVEPKSCDKTHTCPPCPAPELLGGPSVFLFPPKPKDTLMISRTPEVTCVVVDVSHEDPEVKFNWYVDGVEVHNAKTKPREEQYNSTYRVVSVLTVLHQDWLNGKEYKCKVSNKALPAPIEKTISKAKGQPREPQVYTLPPSRDELTKNQVSLTCLVKGFYPSDIAVEWESNGQPENNYKTTPPVLDSDGSFFLYSKLTVDKSRWQQGNVFSCSVMHEALHNHYTQKSLSLSPGKGSSETQANSTTDALNVLLIIVDDLRPSLGCYGDKLVRSPNIDQLASHSLLFQNAFAQQAVCAPSRVSFLTGRRPDTTRLYDFNSYWRVHAGNFSTIPQYFKENGYVTMSVGKVFHPGISSNHTDDSPYSWSFPPYHPSSEKYENTKTCRGPDGELHANLLCPVDVLDVPEGTLPDKQSTEQAIQLLEKMKTSASPFFLAVGYHKPHIPFRYPKEFQKLYPLENITLAPDPEVPDGLPPVAYNPWMDIRQREDVQALNISVPYGPIPVDFQRKIRQSYFASVSYLDTQVGRLLSALDDLQLANSTIIAFTSDHGWALGEHGEWAKYSNFDVATHVPLIFYVPGRTASLPEAGEKLFPYLDPFDSASQLMEPGRQSMDLVELVSLFPTLAGLAGLQVPPRCPVPSFHVELCREGKNLLKHFRFRDLEEDPYLPGNPRELIAYSQYPRPSDIPQWNSDKPSLKDIKIMGYSIRTIDYRYTVWVGFNPDEFLANFSDIHAGELYFVDSDPLQDHNMYNDSQGGDLFQLLMP

SEQ ID NO: 14 - DNA, 3002 bp, Artificial Sequence
  Nucleotide seuquence encoding amino acid sequence of fused protein of the heavy-chain of humanized anti-hTfR antibody No.1 and hI2S, synthetic sequence
acgcgtgccgccaccatgggctggagctggattctgctgttcctcctgagcgtgacagcaggagtgcacagcgaagtgcagctggtcgaatcagggggggggctggtgcagcctggaggcagcctgagactgtcctgcgccgcttctggcttgacctttagcaactacgggatgtcctgggtgcggcaggctcctggcaagggactggagttggtggccaacatcaataccaacggcggaagtacatactatcccgattcagtgaagggccggttcaccatcagcagggacaacgccaagaacagcctgtatctgcagatgaactctctgagggccgaggatacagccgtgtactattgcactaacaaccggtacgacgaggactattggggccagggcaccctggtgacagtgtctagcgcctctaccaagggcccaagcgtgtttcctctggctccatcctctaaatccacctctggcggcacagccgctctgggctgtctggtgaaggattacttcccagagcccgtgacagtgtcttggaacagcggcgccctgacctccggcgtgcacacatttcctgctgtgctgcagagctccggcctgtacagcctgtctagcgtggtgaccgtgccatcctctagcctgggcacccagacatatatctgcaacgtgaatcacaagcccagcaatacaaaggtggataagaaggtggagccaaagtcctgtgacaagacccacacatgccccccttgtcctgctccagagctgctgggaggaccaagcgtgttcctgtttccacccaagcccaaggataccctgatgatctctcggaccccagaggtgacatgcgtggtggtggatgtgagccacgaggaccccgaggtgaagttcaactggtatgtggacggcgtggaggtgcacaatgctaagaccaagcccagggaggagcagtacaactccacctatagagtggtgtctgtgctgacagtgctgcaccaggattggctgaacggcaaggagtataagtgcaaggtgtccaataaggccctgcccgctcctatcgagaagaccatctctaaggccaagggccagcccagagagcctcaggtgtacacactgcctccatcccgggatgagctgaccaagaaccaggtgtctctgacatgtctggtcaagggcttctatccctctgacatcgccgtggagtgggagagcaatggccagcctgagaacaattacaagaccacaccccctgtgctggattccgacggctctttctttctgtatagcaagctgaccgtggacaagtcccggtggcagcagggcaacgtgttcagctgttccgtgatgcacgaagctctgcataatcactatactcagaaatccctgtcactgtcacctggtaaaggatcttccgaaacgcaggccaactcgaccacagatgctctgaacgttcttctcatcatcgtggatgacctgcgcccctccctgggctgttatggggataagctggtgaggtccccaaatattgaccaactggcatcccacagcctcctcttccagaatgcctttgcgcagcaagcagtgtgcgccccgagccgcgtttctttcctcactggcaggagacctgacaccacccgcctgtacgacttcaactcctactggagggtgcacgctggaaacttctccaccatcccccagtacttcaaggagaatggctatgtgaccatgtcggtgggaaaagtctttcaccctgggatatcttctaaccataccgatgattctccgtatagctggtcttttccaccttatcatccttcctctgagaagtatgaaaacactaagacatgtcgagggccagatggagaactccatgccaacctgctttgccctgtggatgtgctggatgttcccgagggcaccttgcctgacaaacagagcactgagcaagccatacagttgttggaaaagatgaaaacgtcagccagtcctttcttcctggccgttgggtatcataagccacacatccccttcagataccccaaggaatttcagaagttgtatcccttggagaacatcaccctggcccccgatcccgaggtccctgatggcctaccccctgtggcctacaacccctggatggacatcaggcaacgggaagacgtccaagccttaaacatcagtgtgccgtatggtccaattcctgtggactttcagcggaaaatccgccagagctactttgcctctgtgtcatatttggatacacaggtcggccgcctcttgagtgctttggacgatcttcagctggccaacagcaccatcattgcatttacctcggatcatgggtgggctctaggtgaacatggagaatgggccaaatacagcaattttgatgttgctacccatgttcccctgatattctatgttcctggaaggacggcttcacttccggaggcaggcgagaagcttttcccttacctcgacccttttgattccgcctcacagttgatggagccaggcaggcaatccatggaccttgtggaacttgtgtctctttttcccacgctggctggacttgcaggactgcaggttccacctcgctgccccgttccttcatttcacgttgagctgtgcagagaaggcaagaaccttctgaagcattttcgattccgtgacttggaagaagatccgtacctccctggtaatccccgtgaactgattgcctatagccagtatccccggccttcagacatccctcagtggaattctgacaagccgagtttaaaagatataaagatcatgggctattccatacgcaccatagactataggtatactgtgtgggttggcttcaatcctgatgaatttctagctaacttttctgacatccatgcaggggaactgtattttgtggattctgacccattgcaggatcacaatatgtataatgattcccaaggtggagaccttttccagttgttgatgccttaagcggccgc

SEQ ID NO: 15 - protein, 980 aa, Artificial Sequence
  Amino acid sequence of fused protein of the heavy-chain of humanized anti-hTfR antibody No.2 and hI2S
QVQLVQSGAEVKKPGASVKVSCKASGYTFTDYVMHWVRQAPGQGLEWIGVISTYYGHGSYNQRFKGRATMTVDKSISTAYMELVRLRSDDTAVYYCVRGGYGSSSLAGNFDVWGQGTTVTVSSASTKGPSVFPLAPSSKSTSGGTAALGCLVKDYFPEPVTVSWNSGALTSGVHTFPAVLQSSGLYSLSSVVTVPSSSLGTQTYICNVNHKPSNTKVDKKVEPKSCDKTHTCPPCPAPELLGGPSVFLFPPKPKDTLMISRTPEVTCVVVDVSHEDPEVKFNWYVDGVEVHNAKTKPREEQYNSTYRVVSVLTVLHQDWLNGKEYKCKVSNKALPAPIEKTISKAKGQPREPQVYTLPPSRDELTKNQVSLTCLVKGFYPSDIAVEWESNGQPENNYKTTPPVLDSDGSFFLYSKLTVDKSRWQQGNVFSCSVMHEALHNHYTQKSLSLSPGKGSSETQANSTTDALNVLLIIVDDLRPSLGCYGDKLVRSPNIDQLASHSLLFQNAFAQQAVCAPSRVSFLTGRRPDTTRLYDFNSYWRVHAGNFSTIPQYFKENGYVTMSVGKVFHPGISSNHTDDSPYSWSFPPYHPSSEKYENTKTCRGPDGELHANLLCPVDVLDVPEGTLPDKQSTEQAIQLLEKMKTSASPFFLAVGYHKPHIPFRYPKEFQKLYPLENITLAPDPEVPDGLPPVAYNPWMDIRQREDVQALNISVPYGPIPVDFQRKIRQSYFASVSYLDTQVGRLLSALDDLQLANSTIIAFTSDHGWALGEHGEWAKYSNFDVATHVPLIFYVPGRTASLPEAGEKLFPYLDPFDSASQLMEPGRQSMDLVELVSLFPTLAGLAGLQVPPRCPVPSFHVELCREGKNLLKHFRFRDLEEDPYLPGNPRELIAYSQYPRPSDIPQWNSDKPSLKDIKIMGYSIRTIDYRYTVWVGFNPDEFLANFSDIHAGELYFVDSDPLQDHNMYNDSQGGDLFQLLMP

SEQ ID NO: 16 - DNA, 3023 bp, Artificial Sequence
  Nucleotide seuquence encoding amino acid sequence of fused protein of the heavy-chain of humanized anti-hTfR antibody No.2 and hI2S, synthetic sequence
acgcgtgccgccaccatgggctggagctggattctgctgttcctcctgagcgtgacagcaggagtgcacagccaggtgcagctggtccagtcaggagccgaagtgaaaaagcccggagcctcagtcaaagtgtcttgtaaagcatcaggttatacatttacagactacgtcatgcactgggtgaggcaggcacctggacagggtctggaatggatcggcgtgatctccacttactatggccatggaagctacaaccagagattcaagggcagggcgacaatgactgtagacaaatcaatttccactgcttatatggagctggtaaggctgcggtccgacgataccgctgtgtactattgcgtacgaggaggatacggctccagctctctggctggtaatttcgatgtgtgggggcagggtaccacagtcaccgtgagttcagcaagcacaaagggcccatctgtgtttccactggccccctccagcaaaagcacctctgggggtacagccgctctgggatgtctggtgaaggattatttcccagagccagtcaccgtgtcctggaacagcggagccctgacatctggagtccacacttttccagctgtgctgcagtctagtgggctgtactccctgtcatccgtggtcactgtccccagctctagtctgggtacccagacatatatctgcaacgtgaatcacaagccatctaataccaaagtcgacaagaaagtggaacccaagtcctgtgataaaactcatacctgccccccttgtcctgcaccagagctgctgggaggaccatccgtgttcctgtttccacccaagcctaaagacaccctgatgattagccgaactcccgaagtcacctgcgtggtcgtggacgtgtctcacgaggaccctgaagtcaagtttaactggtacgtggatggcgtcgaggtgcataatgctaagacaaaaccccgagaggaacagtacaacagtacatatcgtgtcgtgtcagtgctgaccgtcctgcatcaggactggctgaacgggaaggaatataagtgcaaagtgtccaataaggcactgcccgcccctatcgagaaaaccattagcaaggccaaaggacagcctagggaaccacaggtgtacacactgcctccatcccgggacgagctgactaagaaccaggtcagcctgacctgtctggtgaaaggcttctatccttcagatatcgctgtggagtgggaaagtaatggacagccagagaacaattacaagactaccccccctgtgctggactctgatgggagtttctttctgtattctaagctgaccgtggataaaagtcggtggcagcagggtaatgtctttagttgttcagtgatgcacgaagcactgcacaaccactacacccagaaatcactgtcactgtcaccagggaaaggatcttccgaaacgcaggccaactcgaccacagatgctctgaacgttcttctcatcatcgtggatgacctgcgcccctccctgggctgttatggggataagctggtgaggtccccaaatattgaccaactggcatcccacagcctcctcttccagaatgcctttgcgcagcaagcagtgtgcgccccgagccgcgtttctttcctcactggcaggagacctgacaccacccgcctgtacgacttcaactcctactggagggtgcacgctggaaacttctccaccatcccccagtacttcaaggagaatggctatgtgaccatgtcggtgggaaaagtctttcaccctgggatatcttctaaccataccgatgattctccgtatagctggtcttttccaccttatcatccttcctctgagaagtatgaaaacactaagacatgtcgagggccagatggagaactccatgccaacctgctttgccctgtggatgtgctggatgttcccgagggcaccttgcctgacaaacagagcactgagcaagccatacagttgttggaaaagatgaaaacgtcagccagtcctttcttcctggccgttgggtatcataagccacacatccccttcagataccccaaggaatttcagaagttgtatcccttggagaacatcaccctggcccccgatcccgaggtccctgatggcctaccccctgtggcctacaacccctggatggacatcaggcaacgggaagacgtccaagccttaaacatcagtgtgccgtatggtccaattcctgtggactttcagcggaaaatccgccagagctactttgcctctgtgtcatatttggatacacaggtcggccgcctcttgagtgctttggacgatcttcagctggccaacagcaccatcattgcatttacctcggatcatgggtgggctctaggtgaacatggagaatgggccaaatacagcaattttgatgttgctacccatgttcccctgatattctatgttcctggaaggacggcttcacttccggaggcaggcgagaagcttttcccttacctcgacccttttgattccgcctcacagttgatggagccaggcaggcaatccatggaccttgtggaacttgtgtctctttttcccacgctggctggacttgcaggactgcaggttccacctcgctgccccgttccttcatttcacgttgagctgtgcagagaaggcaagaaccttctgaagcattttcgattccgtgacttggaagaagatccgtacctccctggtaatccccgtgaactgattgcctatagccagtatccccggccttcagacatccctcagtggaattctgacaagccgagtttaaaagatataaagatcatgggctattccatacgcaccatagactataggtatactgtgtgggttggcttcaatcctgatgaatttctagctaacttttctgacatccatgcaggggaactgtattttgtggattctgacccattgcaggatcacaatatgtataatgattcccaaggtggagaccttttccagttgttgatgccttaagcggccgc

SEQ ID NO: 17 - protein, 975 aa, Artificial Sequence
  Amino acid sequence of fused protein of the heavy-chain of humanized anti-hTfR antibody No. 3 and hI2S
EVQLVQSGAEVKKPGESLKISCKGSGYSFMNYWLGWVRQMPGKGLEWIGDIYPGGDYPTYSEKFKVKAIISADTSISTVYLQLSSLKASDTAMYFCARSGNYDEVAYWGQGTLVTVSSASTKGPSVFPLAPSSKSTSGGTAALGCLVKDYFPEPVTVSWNSGALTSGVHTFPAVLQSSGLYSLSSVVTVPSSSLGTQTYICNVNHKPSNTKVDKKVEPKSCDKTHTCPPCPAPELLGGPSVFLFPPKPKDTLMISRTPEVTCVVVDVSHEDPEVKFNWYVDGVEVHNAKTKPREEQYNSTYRVVSVLTVLHQDWLNGKEYKCKVSNKALPAPIEKTISKAKGQPREPQVYTLPPSRDELTKNQVSLTCLVKGFYPSDIAVEWESNGQPENNYKTTPPVLDSDGSFFLYSKLTVDKSRWQQGNVFSCSVMHEALHNHYTQKSLSLSPGKGSSETQANSTTDALNVLLIIVDDLRPSLGCYGDKLVRSPNIDQLASHSLLFQNAFAQQAVCAPSRVSFLTGRRPDTTRLYDFNSYWRVHAGNFSTIPQYFKENGYVTMSVGKVFHPGISSNHTDDSPYSWSFPPYHPSSEKYENTKTCRGPDGELHANLLCPVDVLDVPEGTLPDKQSTEQAIQLLEKMKTSASPFFLAVGYHKPHIPFRYPKEFQKLYPLENITLAPDPEVPDGLPPVAYNPWMDIRQREDVQALNISVPYGPIPVDFQRKIRQSYFASVSYLDTQVGRLLSALDDLQLANSTIIAFTSDHGWALGEHGEWAKYSNFDVATHVPLIFYVPGRTASLPEAGEKLFPYLDPFDSASQLMEPGRQSMDLVELVSLFPTLAGLAGLQVPPRCPVPSFHVELCREGKNLLKHFRFRDLEEDPYLPGNPRELIAYSQYPRPSDIPQWNSDKPSLKDIKIMGYSIRTIDYRYTVWVGFNPDEFLANFSDIHAGELYFVDSDPLQDHNMYNDSQGGDLFQLLMP

SEQ ID NO: 18 - DNA, 3008 bp, Artificial Sequence
  Nucleotide seuquence encoding amino acid sequence of fused protein of the heavy-chain of humanized anti-hTfR antibody No.3 and hI2S, synthetic sequence
acgcgtgccgccaccatgggctggagctggattctgctgttcctcctgagcgtgacagcaggagtgcacagcgaggtgcaactagtgcagtctggagcagaggtgaaaaagcccggggagtctctgaagatcagctgtaagggttctggatacagctttatgaactactggctgggatgggtgcgccagatgcccgggaaaggcctggagtggattggggacatctaccccggcggagactaccctacatacagcgagaagttcaaggtcaaggccatcatctcagccgacacgtccatcagcaccgtctacctgcagttgagcagcctgaaggcctcggacaccgccatgtatttctgtgcgagatcaggcaattacgacgaagtggcctactggggccaaggaaccctggtcaccgtctcctcagctagcaccaagggcccatcggtcttccccctggcaccctcctccaagagcacctctgggggcacagcggccctgggctgcctggtcaaggactacttccccgaaccggtgacggtgtcgtggaactcaggcgccctgaccagcggcgtgcacaccttcccggctgtcctacagtcctcaggactctactccctcagcagcgtggtgaccgtgccctccagcagcttgggcacccagacctacatctgcaacgtgaatcacaagcccagcaacaccaaggtggacaagaaagttgagcccaaatcttgtgacaaaactcacacgtgcccaccgtgcccagcacctgaactcctggggggtccgtcagtcttcctcttccccccaaaacccaaggacaccctcatgatctcccggacccctgaggtcacatgcgtggtggtggacgtgagccacgaagaccctgaggtcaagttcaactggtacgtggacggcgtggaggtgcataatgccaagacaaagccgcgggaggagcagtacaacagcacgtaccgggtggtcagcgtcctcaccgtcctgcaccaggactggctgaatggcaaggagtacaagtgcaaggtctccaacaaagccctcccagcccccatcgagaaaaccatctccaaagccaaagggcagccccgagaaccacaggtgtacaccctgcccccatcccgggatgagctgaccaagaaccaggtcagcctgacctgcctggtcaaaggcttctatcccagcgacatcgccgtggagtgggagagcaatgggcagccggagaacaactacaagaccacgcctcccgtgctggactccgacggctccttcttcctctacagcaagctcaccgtggacaagagcaggtggcagcaggggaacgtcttctcatgctccgtgatgcatgaggctctgcacaaccactacacgcagaagagcctctccctgtctccgggtaaaggatcttccgaaacgcaggccaactcgaccacagatgctctgaacgttcttctcatcatcgtggatgacctgcgcccctccctgggctgttatggggataagctggtgaggtccccaaatattgaccaactggcatcccacagcctcctcttccagaatgcctttgcgcagcaagcagtgtgcgccccgagccgcgtttctttcctcactggcaggagacctgacaccacccgcctgtacgacttcaactcctactggagggtgcacgctggaaacttctccaccatcccccagtacttcaaggagaatggctatgtgaccatgtcggtgggaaaagtctttcaccctgggatatcttctaaccataccgatgattctccgtatagctggtcttttccaccttatcatccttcctctgagaagtatgaaaacactaagacatgtcgagggccagatggagaactccatgccaacctgctttgccctgtggatgtgctggatgttcccgagggcaccttgcctgacaaacagagcactgagcaagccatacagttgttggaaaagatgaaaacgtcagccagtcctttcttcctggccgttgggtatcataagccacacatccccttcagataccccaaggaatttcagaagttgtatcccttggagaacatcaccctggcccccgatcccgaggtccctgatggcctaccccctgtggcctacaacccctggatggacatcaggcaacgggaagacgtccaagccttaaacatcagtgtgccgtatggtccaattcctgtggactttcagcggaaaatccgccagagctactttgcctctgtgtcatatttggatacacaggtcggccgcctcttgagtgctttggacgatcttcagctggccaacagcaccatcattgcatttacctcggatcatgggtgggctctaggtgaacatggagaatgggccaaatacagcaattttgatgttgctacccatgttcccctgatattctatgttcctggaaggacggcttcacttccggaggcaggcgagaagcttttcccttacctcgacccttttgattccgcctcacagttgatggagccaggcaggcaatccatggaccttgtggaacttgtgtctctttttcccacgctggctggacttgcaggactgcaggttccacctcgctgccccgttccttcatttcacgttgagctgtgcagagaaggcaagaaccttctgaagcattttcgattccgtgacttggaagaagatccgtacctccctggtaatccccgtgaactgattgcctatagccagtatccccggccttcagacatccctcagtggaattctgacaagccgagtttaaaagatataaagatcatgggctattccatacgcaccatagactataggtatactgtgtgggttggcttcaatcctgatgaatttctagctaacttttctgacatccatgcaggggaactgtattttgtggattctgacccattgcaggatcacaatatgtataatgattcccaaggtggagaccttttccagttgttgatgccttaagcggccgc

SEQ ID NO: 19 - protein, 5 aa, Artificial Sequence
  Amino acid sequence of an exemplified linker 1
GGGGS

SEQ ID NO: 20 - protein, 6 aa, Artificial Sequence
  Amino acid sequence of an exemplified linker 2
GGGGGS

SEQ ID NO: 21 - protein, 6 aa, Artificial Sequence
  Amino acid sequence of an exemplified linker 3
SGGGGG

SEQ ID NO: 22 - protein, 760 aa, Homo sapiens
MMDQARSAFSNLFGGEPLSYTRFSLARQVDGDNSHVEMKLAVDEEENADNNTKANVTKPKRCSGSICYGTIAVIVFFLIGFMIGYLGYCKGVEPKTECERLAGTESPVREEPGEDFPAARRLYWDDLKRKLSEKLDSTDFTGTIKLLNENSYVPREAGSQKDENLALYVENQFREFKLSKVWRDQHFVKIQVKDSAQNSVIIVDKNGRLVYLVENPGGYVAYSKAATVTGKLVHANFGTKKDFEDLYTPVNGSIVIVRAGKITFAEKVANAESLNAIGVLIYMDQTKFPIVNAELSFFGHAHLGTGDPYTPGFPSFNHTQFPPSRSSGLPNIPVQTISRAAAEKLFGNMEGDCPSDWKTDSTCRMVTSESKNVKLTVSNVLKEIKILNIFGVIKGFVEPDHYVVVGAQRDAWGPGAAKSGVGTALLLKLAQMFSDMVLKDGFQPSRSIIFASWSAGDFGSVGATEWLEGYLSSLHLKAFTYINLDKAVLGTSNFKVSASPLLYTLIEKTMQNVKHPVTGQFLYQDSNWASKVEKLTLDNAAFPFLAYSGIPAVSFCFCEDTDYPYLGTTMDTYKELIERIPELNKVARAAAEVAGQFVIKLTHDVELNLDYERYNSQLLSFVRDLNQYRADIKEMGLSLQWLYSARGDFFRATSRLTTDFGNAEKTDRFVMKKLNDRVMRVEYHFLSPYVSPKESPFRHVFWGSGSHTLPALLENLKLRKQNNGAFNETLFRNQLALATWTIQGAANALSGDVWDIDNEF

SEQ ID NO: 23 - protein, 107 aa, Artificial Sequence
  Amino acid sequence of the light-chain variable region of humanized anti-hTfR antibody No.1
DIQVTQSPSFLSASVGDRVTITCKASQDVNSAVAWFQQKPGKAPKLLIYWTSTRHTGVPDRFSGSGSGTVYTLTISSLQPEDFATYYCQQHYSTPRTFGGGTKVEIK

SEQ ID NO: 24 - protein, 116 aa, Artificial Sequence
  Amino acid sequence of the heavy-chain variable region of humanized anti-hTfR antibody No.1
EVQLVESGGGLVQPGGSLRLSCAASGLTFSNYGMSWVRQAPGKGLELVANINTNGGSTYYPDSVKGRFTISRDNAKNSLYLQMNSLRAEDTAVYYCTNNRYDEDYWGQGTLVTVSS

SEQ ID NO: 25 - protein, 107 aa, Artificial Sequence
  Amino acid sequence of the light-chain variable region of humanized anti-hTfR antibody No.2
EIVLTQSPDFQSVTPKEKVTITCRASQSISNNLQWYQQKPDQSPKLLIKYASQSISGIPSRFSGSGSGTDFTLTINSLEAEDAATYLCQQSNSWPRTFGQGTKVEIK

SEQ ID NO: 26 - protein, 120 aa, Artificial Sequence
  Amino acid sequence of the heavy-chain variable region of humanized anti-hTfR antibody No.2
QVQLVQSGAEVKKPGASVKVSCKASGYTFTDYVMHWVRQAPGQGLEWIGVISTYYGHGSYNQRFKGRATMTVDKSISTAYMELVRLRSDDTAVYYCVRGGYGSSSLAGNFDVWGQGTTVT

SEQ ID NO: 27 - protein, 112 aa, Artificial Sequence
  Amino acid sequence of the light-chain variable region of humanized anti-hTfR antibody No.3
DIVMTQTPLSLSVTPGQPASISCRSSQSLVHSNGNTYLHWYLQKPGQSPQLLIYKVSNRFSGVPDRFSGSGSGTDFTLKISRVEAEDVGVYYCSQSTHVPWTFGQGTKVEIK

SEQ ID NO: 28 - protein, 118 aa, Artificial Sequence
  Amino acid sequence of the heavy-chain variable region of humanized anti-hTfR antibody No.3
EVQLVQSGAEVKKPGESLKISCKGSGYSFTNYWLGWVRQMPGKGLEWMGDIYPGGDYPTYSEKFKVQVTISADKSISTAYLQWSSLKASDTAMYYCARSGNYDEVAYWGQGTLVTVSS

SEQ ID NO: 29 - protein, 6 aa, Artificial Sequence
  Amino acid sequence 1 of CDR1 in the light chain of anti-hTfR antibody No. 1
QDVNSA

SEQ ID NO: 30 - protein, 11 aa, Artificial Sequence
  Amino acid sequence 2 of CDR1 in the light chain of anti-hTfR antibody No. 1
KASQDVNSAVA

SEQ ID NO: 31 - protein, 6 aa, Artificial Sequence
  Amino acid sequence 1 of CDR2 in the light chain of anti-hTfR antibody No. 1
WTSTRH

SEQ ID NO: 32 - protein, 7 aa, Artificial Sequence
  Amino acid sequence 2 of CDR2 in the light chain of anti-hTfR antibody No. 1
WTSTRHT

SEQ ID NO: 33 - protein, 9 aa, Artificial Sequence
  Amino acid sequence of CDR3 in the light chain of anti-hTfR antibody No. 1
QQHYSTPRT

SEQ ID NO: 34 - protein, 5 aa, Artificial Sequence
  Amino acid sequence 1 of CDR1 in the heavy chain of anti-hTfR antibody No. 1
NYGMS

SEQ ID NO: 35 - protein, 8 aa, Artificial Sequence
  Amino acid sequence 2 of CDR1 in the heavy chain of anti-hTfR antibody No. 1
GLTFSNYG

SEQ ID NO: 36 - protein, 8 aa, Artificial Sequence
  Amino acid sequence 1 of CDR2 in the heavy chain of anti-hTfR antibody No. 1
INTNGGST

SEQ ID NO: 37 - protein, 17 aa, Artificial Sequence
  Amino acid sequence 2 of CDR2 in the heavy chain of anti-hTfR antibody No. 1
NINTNGGSTYYPDSVKG

SEQ ID NO: 38 - protein, 7 aa, Artificial Sequence
  Amino acid sequence 1 of CDR3 in the heavy chain of anti-hTfR antibody No. 1
NRYDEDY

SEQ ID NO: 39 - protein, 9 aa, Artificial Sequence
  Amino acid sequence 2 of CDR3 in the heavy chain of anti-hTfR antibody No. 1
TNNRYDEDY

SEQ ID NO: 40 - protein, 6 aa, Artificial Sequence
  Amino acid sequence 1 of CDR1 in the light chain of anti-hTfR antibody No. 2
QSISNN

SEQ ID NO: 41 - protein, 11 aa, Artificial Sequence
  Amino acid sequence 2 of CDR1 in the light chain of anti-hTfR antibody No. 2
RASQSISNNLQ

SEQ ID NO: 42 - protein, 6 aa, Artificial Sequence
  Amino acid sequence 1 of CDR2 in the light chain of anti-hTfR antibody No. 2
YASQSI

SEQ ID NO: 43 - protein, 7 aa, Artificial Sequence
  Amino acid sequence 2 of CDR2 in the light chain of anti-hTfR antibody No. 2
YASQSIS

SEQ ID NO: 44 - protein, 9 aa, Artificial Sequence
  Amino acid sequence of CDR3 in the light chain of anti-hTfR antibody No. 2
QQSNSWPRT

SEQ ID NO: 45 - protein, 5 aa, Artificial Sequence
  Amino acid sequence 1 of CDR1 in the heavy chain of anti-hTfR antibody No. 2
DYVMH

SEQ ID NO: 46 - protein, 8 aa, Artificial Sequence
  Amino acid sequence 2 of CDR1 in the heavy chain of anti-hTfR antibody No. 2
GYTFTDYV

SEQ ID NO: 47 - protein, 8 aa, Artificial Sequence
  Amino acid sequence 1 of CDR2 in the heavy chain of anti-hTfR antibody No. 2
ISTYYGHG

SEQ ID NO: 48 - protein, 17 aa, Artificial Sequence
  Amino acid sequence 2 of CDR2 in the heavy chain of anti-hTfR antibody No. 2
VISTYYGHGSYNQRFKG

SEQ ID NO: 49 - protein, 14 aa, Artificial Sequence
  Amino acid sequence 1 of CDR3 in the heavy chain of anti-hTfR antibody No. 2
GGYGSSSLAGNFDV

SEQ ID NO: 50 - protein, 16 aa, Artificial Sequence
  Amino acid sequence 2 of CDR3 in the heavy chain of anti-hTfR antibody No. 2
VRGGYGSSSLAGNFDV

SEQ ID NO: 51 - protein, 11 aa, Artificial Sequence
  Amino acid sequence 1 of CDR1 in the light chain of anti-hTfR antibody No. 3
QSLVHSNGNTY

SEQ ID NO: 52 - protein, 16 aa, Artificial Sequence
  Amino acid sequence 2 of CDR1 in the light chain of anti-hTfR antibody No. 3
RSSQSLVHSNGNTYLH

SEQ ID NO: 53 - protein, 6 aa, Artificial Sequence
  Amino acid sequence 1 of CDR2 in the light chain of anti-hTfR antibody No. 3
KVSNRF

SEQ ID NO: 54 - protein, 7 aa, Artificial Sequence
  KVSNRFS
KVSNRFS

SEQ ID NO: 55 - protein, 9 aa, Artificial Sequence
  Amino acid sequence of CDR3 in the light chain of anti-hTfR antibody No. 3
SQSTHVPWT

SEQ ID NO: 56 - protein, 5 aa, Artificial Sequence
  Amino acid sequence 1 of CDR1 in the heavy chain of anti-hTfR antibody No. 3
NYWLG

SEQ ID NO: 57 - protein, 8 aa, Artificial Sequence
  Amino acid sequence 2 of CDR1 in the heavy chain of anti-hTfR antibody No. 3
GYSFTNYW

SEQ ID NO: 58 - protein, 8 aa, Artificial Sequence
  Amino acid sequence 1 of CDR2 in the heavy chain of anti-hTfR antibody No. 3
IYPGGDYP

SEQ ID NO: 59 - protein, 17 aa, Artificial Sequence
  Amino acid sequence 2 of CDR2 in the heavy chain of anti-hTfR antibody No. 3
DIYPGGDYPTYSEKFKV

SEQ ID NO: 60 - protein, 9 aa, Artificial Sequence
  Amino acid sequence 1 of CDR3 in the heavy chain of anti-hTfR antibody No. 3
SGNYDEVAY

SEQ ID NO: 61 - protein, 11 aa, Artificial Sequence
  Amino acid sequence 2 of CDR3 in the heavy chain of anti-hTfR antibody No. 3
ARSGNYDEVAY